European Patent Specification EP 3 669 003 B1, published May 10, 2023. Title: PDCD1 as epigenetic marker for the identification of immune cells, in particular PD1+ cells. Applicant: Epiontis GmbH. The sequence listing filed with the application follows.

SEQUENCE LISTING (13 sequences)

SEQ ID NO: 1 - DNA, 11680 bp, Homo sapiens
agtagcaatgtggagagaccatcaggcagccctggcctcagtggccgcagtcccctggctccacgctgggcccaccccaccaggtctcctctcccatggcccaggggccttcagtgggactgagaggaggagggaaggagagtgggtgacagggaagaactgcagggagagaggagaggggtgggagaaggagaaggaaggaaggggtaggatggaagctgggtttctccctgtgcccgccccctactccaggacatgtgtccaagccctggcaggtggaattttgggggcagggccttggtggtgaggagaccttccaggggtctgatagcatctcccatctcagagcccacctcctgggcccagcctcccctccagcccacacagtggcattcccagtcctcagaggacagcttcgtcccacaaagctcagagccttgaggaaggcccactgctgccctggaacagagacagcattcaacagaggttggaacaaggctctacagggctgggggcagagggaggttctgtccagaatctgccttcaggacaagtacagccagcaggggcagcttagccacttatccactgcctgggcgaggcacagggctatggaggcacctaccaaccaacagttctccagccccagagccccagcccctgaggcacaagggtgggtgtgccaggagacagttgctgcgggccaccttagctgtctggcagcacagtgggtgctgccaggctccctgggggccccccgccaagcccacctggccagctgggcccccccccacctccccaccaagccacccacacagcctcacatctctgagacccgggagtggccctttgttcataaacgagagcttcctcgccgtggccgcgcctcgcagacatcatctttgatgctctttttccactgtttcggtgctttaatgttttcccttcagagccgggccgagtgtctctcggagccaggcagccgcgccagctgtcaggcggtttctagcctcgcttcggttattttaagctgatgagcctgacgcatctcatcactaatatcagcagtttcatttctcctgttttccattcgctgtaataaaatgctcagcacagaatacaaggagataagcaagccatttcacaaacgccgggccgccagccaggcccaggcactggaccccctgaaccaccccaccctggcacgagtgggctggagggcagggccccggggaagaaggtcaaggctggaaggggaggtcagcctcacagccagcccctgccaccgccccagcccccccgtcaggctgttgcaggcatcacacggtggaaagatctggaactgtggccatggtgtgaggccatccacaaggtggaagctttgagggggagccgattagccatggacagttgtcattcagtagggtcacctgtgccccagcgaagggggatgggccgggaaggcagaggccaggcacctgcccccagcaggggcagaggctgtgggcagccgggaggctcccagaggctccgacagaatgggagtggggttgagcccacccctcactgcagcccaggaacctgagcccagagggggccacccaccttccccaggcagggaggcccggcccccagggagatgggggggatgggggaggagaagggcctgcccccacccggcagcctcaggaggggcagctcgggcgggatatggaaagaggccacagcagtgagcagagacacagaggaggaaggggccctgagctggggagacccccacggggtagggcgtgggggccacgggcccacctcctccccatctcctctgtctccctgtctctgtctctctctccctcccccaccctctccccagtcctaccccctcctcacccctcctcccccagcactgcctctgtcactctcgcccacgtggatgtggaggaagagggggcgggagcaaggggcgggcaccctcccttcaacctgacctgggacagtttcccttccgctcacctccgcctgagcagtggagaaggcggcactctggtggggctgctccaggcatgcagatcccacaggcgccctggccagtcgtctgggcggtgctacaactgggctggcggccaggatggttcttaggtaggtggggtcggcggtcaggtgtcccagagccaggggtctggagggaccttccaccctcagtccctggcaggtcggggggtgctgaggcgggcctggccctggcagcccaggggtcccggagcgaggggtctggagggacctttcactctcagtccctggcaggtcggggggtgctgtggcaggcccagccttggcccccagctctgccccttaccctgagctgtgtggctttgggcagctcgaactcctgggttcctctctgggccccaactcctcccctggcccaagtcccctctttgctcctgggcaggcaggacctctgtcccctctcagccggtccttggggctgcgtgtttctgtagaatgacgggtcaggctggccagaaccccaaaccttggccgtggggagtctgcgtggcggctctgccttgcccaggcatccttggtcctcactcgagttttcctaaggatgggatgagccccatgtgggactaaccttggctttacgacgtcaaagtttagatgagctggtgatatttttctcattatatccaaagtgtacctgttcgagtgaggacagttcttctgtctccaggatccctcctgggtggggattgtgcccgcctgggtctctgcccagattccagggctctccccgagccctgttcagaccatccgtgggggaggccttggcctcactctcccggatcgaggagagagggagcctcttcctgggctgcccgtgaccctgggccctctgtgtacactgtgaccacagcccgctcctggaccctctgtgcccggctggccctctgtgcccagccagcctgcacctggggatgccaaggcctggggagggtggtttcacccaggccaagcctaagacagtccctctgggccctgctgggtaccggggtgtgacaccactgggaggacaagatgaggggcacccctggggccgccctgacaccccctcgaggctcctgccccgggggtcctggtgccccttcactgtggcaggcgactgggggttccccacctcggcccctctcccggggcctgctccccggcacctgaggcagcatccttgtcagggccgtgccttcctgcctcagcgccacctcttaaggttggcccgtgggtcactcaggactcagaactggagattctgggcaaaaggcaaagagcaaagggccaaaaggcatcccagggagacgactgcgggggaaccagagggcagaggggcgctcgtcacaggggagggggagctgagcgaggcaggaggggagccgagcctctccccccgtgtcccggctcttcaggcacgccctcgggacgccaccctccccgacccaggcgggaaagataagagcaaggtgtccgcagcctgacactcgtgcctcaggtgcccgcgcttgtgccggacaagactctcacaggtggcatgcctcggtttccccactggtaacagcacagggcactcagcaaggcgcagtgggcatgactggggtcctgtgggtcctgacccagatgtggccaccccggccgcagtggtcttcattccaggatgcctcttttccctcctgatctattcactgcgttcgccattcggtcattcccggggccaccactcccacctcaggtgtgtgcttcccttgtgttttatgagatatccccaacccggctgcttattggccccgtccgagggcaggagcataaataagagcctctgctttggcgtgggaccactgtgagctccagtcagcgctgccactgctgagctctgggccttcgacaggacttggccccttactgacttctccgtgtgctttgggtcatgggtgaggacgcctcctggcaaggctgcgtcctgaggattaaatcgggtcatctgtgaaaactacccagcccagcccctgacacttttttgtttgtttcttttagtgacagggtcttgctctgtcacccaggctggagtgcagtggtgtgatctcggctcactcgacctccggggctcaagcaattctcccacctctgcctccagagtagctgggactataggcacgtgccaccctgccaggctaatttcttccattttttttagagacagggtctcgctatgttccccaggctgggctcaaatggtcctcccacctcagcctccccaagtactgggattacaggcataagccactgcatctggcctccatgacacatatttttaaagtctgatttttaaagtcaaacttttgaagtcagattttaaacggactattttgaaaaatatacaaaaacgtttaaaaacaatgaatatccctcacctagaatcaataactaagaatattgacacatttgctttggggactgggcggctggagctgccatgacaaagctccgccgaccgagtggcttttaaacagagcctgccctctcgccgactgagggctggacgtgcaggatggagctccgcagggtcggctcccctgtgctctgaggggctctgctcagcctctcccggctgtggcttaaaaacagagcctgtcctcccgccgtggggggctggacatgcaggaccgaggggccacagggtcggctccctgtgctccgagagggctctgctcagcttctcctggctggggggttttgtggccaccctctgtgttcctgggttcagaagcatcccccaggctctgccttcatctctgcacgggtgactctgtacaggaagccaggcctgctggtcaatggccacccagccctgtgccctcatcttacctagtcccagctgccgtcaccctattcctaataaggccgccttctgaggtcatggggttaggacttccacataggaatctgtggggacacggttcggcccacagcccttcccacctccacacacacacacgactgtgaggagttggaagacctcactcctcacccctgccaggtcctctagggacaagctcgctgtcctcatcccagcacagcccgtgggacggtttccttgtccctaatgggaccacggtcagagatgccgggtctggtctgggccagcaggttcctccgcccggggcaggcagccttcttctgtgcgcttctggaaagcaatgtcctgtaatgcggtctctctgcgggagcacccccaccgccacctcacaggcctgttccacagccccgggatgggctctgtctccctcctgaccctgcatagggcacagccctctctcatcaacccacgatcctacgtggatccgagagggagcacctggggaaacaatggaatcccatagaaacaccccaaatctaacttgatccaggaccagccagtggtcacttctgaatattcaccttcctagtagacactaccagccaagggaggccaggaagccttcctggaggaggtggcctgaggactggggtgaggcaggccctgcgtgggggtcgccacccagcacccccacactgggtgggagccagtctctgagactggctgggggaggtgggagagggggctgcttgaactgcagacaccgaggtctagcccccaccccacccagccagttggtggaggcaggggaggccgaggggcccagctggacctgctccccggggtggattccaaaataggggggttggggggggcggaacaggagcccagggtcctggcttgaggcccagtggctgagggctggtgcaagccagacaggaaaagggttgagcctgtcagcgccagcacagatcaagtcaggagcaggtccctccaccaatgtgtgcaaataaatagcagctaagtttccagttacaagaacaatgcacagatggtcccagggacattgcggtgtggacacacagcggccattgtcctgtcgccagcacctcgccctacagctggggggtcccttagcacttcctagccatgcagggtccctgctcacagtacccgtgatgacttctgttcctcacctgcctgtctgtcccgacagctgcatggcagccctggcctgggagatggagaccccgaggggctgcctgcggtggtggggcccctgggtccccactgcattcccagaaacccagagggcagggcatttcccctgctctgtgccgagtccacccagccccagcctaggcccagtaagggctgcagcccaccctgtcccaggctgcctcccaggagccctcttggccctgatgccagaagcccatcttcctccattcaggcaggtctctgagtgccctggcctggctgcctgctggccctgagagtcacactaccccacagccctccttggtcaaaatccactctggagtggctggaagattccccgggcccacgccgcacacgcctatgcagggagcttcccctggccggccggcagacaagggcggtctcagagagggggctcacctcagcagccccttgtgtagctggccctcgcccctgccacctctgggaacaccaccaggaagctgggggacaggcacgcaggtgaaggaggcgagcgcttgtcagccgggaggccatgggcacagagggaacagggacaccctgggtggcctcaaggtcacttcaaacccctcactcgtcccctgggagggtgcccagtgaggttggcactaggagttggtcctggtcacatgacagacccacccacctctggtgtccagccagcacgccgtgggccagcctggctgcagggacacgagggcagcagccccctcctcctctgagctggttgctccttgagtcatcaccaccgcctgccacggaggccgcctgtcccaggaagcagagggaccgcagctgtggcaaccagggcctggtctctgtgtcacctcgctggggggccgtgcccaggcctgagacggaactgagtgacagtgcactgggtctgacagtgtggggctggcgccatgtttggggaaccctgtggcatgggacctgtgggtgagccgggaaaatcaccccgttgcatggcatctcgggcctggatcttaagcgcctgtgttggtgcctccgcctggcggaagagccgcgacccccacgttgccatgcgggtatcccaagccctgaccctggcaggcatatgtttcaggaggtccttgtcttgggagcccagggtcgggggccccgtgtctgtccacatccgagtcaatggcccatctcgtctctgaagcatctttgctgtgagctctagtccccactgtcttgctggaaaatgtggaggccccactgcccactgcccagggcagcaatgcccataccacgtggtcccagctccgagcttgtcctgaaaagggggcaaagactggaccctgagcctgccaaggggccacactcctcccagggctggggtctccatgggcagccccccacccacccagaccagttacactcccctgtgccagagcagtgcagacaggaccaggccaggatgcccaagggtcaggggctggggatgggtagcccccaaacagccctttctgggggaactggcctcaacggggaagggggtgaaggctcttagtaggaaatcagggagacccaagtcagagccaggtgctgtgcagaagctgcagcctcacgtagaaggaagaggctctgcagtggaggccagtgcccatccccgggtggcagaggccccagcagagacttctcaatgacattccagctggggtggcccttccagagcccttgctgcccgagggatgtgagcaggtggccggggaggctttgtggggccacccagccccttcctcacctctctccatctctcagactccccagacaggccctggaacccccccaccttctccccagccctgctcgtggtgaccgaaggggacaacgccaccttcacctgcagcttctccaacacatcggagagcttcgtgctaaactggtaccgcatgagccccagcaaccagacggacaagctggccgccttccccgaggaccgcagccagcccggccaggactgccgcttccgtgtcacacaactgcccaacgggcgtgacttccacatgagcgtggtcagggcccggcgcaatgacagcggcacctacctctgtggggccatctccctggcccccaaggcgcagatcaaagagagcctgcgggcagagctcagggtgacaggtgcggcctcggaggccccggggcaggggtgagctgagccggtcctggggtgggtgtcccctcctgcacaggatcaggagctccagggtcgtagggcagggaccccccagctccagtccagggctctgtcctgcacctggggaatggtgaccggcatctctgtcctctagctctggaagcaccccagcccctctagtctgccctcacccctgaccctgaccctccaccctgaccccgtcctaacccctgacctttgtgcccttccagagagaagggcagaagtgcccacagcccaccccagcccctcacccaggccagccggccagttccaaaccctggtggttggtgtcgtgggcggcctgctgggcagcctggtgctgctagtctgggtcctggccgtcatctgctcccgggccgcacgaggtaacgtcatcccagcccctcggcctgccctgccctaaccctgctggcggccctcactcccgcctccccttcctccacccttccctcaccccaccccacctccccccatctccccgccaggctaagtccctgatgaaggcccctggactaagacccccccacctaggagcacggctcagggtcggcctggtgaccccaagtgtgtttctctgcagggacaataggagccaggcgcaccggccagcccctggtgagtctcactcttttcctgcatgatccactgtgccttccttcctgggtgggcagaggtggaaggacaggctgggaccacacggcctgcaggactcacattctattatagccaggaccccacctccccagcccccaggcagcaacctcaatccctaaagccatgatctggggccccagcccacctgcggtctccgggggtgcccggcccatgtgtgtgcctgcctgcggtctccaggggtgcctggcccacgcgtgtgcccgcctgcggtctctgggggtgcccggcccacatatgtgcctgcctgcggtctccaggtgtgcccggcccatgcgtgtgcccacctgcgagggcgtggggtgggcttggtcatttcttatcttacattggagacaggagagcttgaaaagtcacattttggaatcctaaatctgcaagaatgccagggacatttcagagggggacattgagccagagaggaggggtggtgtccccagatcacacagagggcagtggtgggacagctcagggtaagcagctcgtagtggggggcccaggttcggtgccggtactgcagccaggctgtggagccgcgggcctccttcctgcggtgggccgtggggctgactccctctccctttctcctcaaagaaggaggacccctcagccgtgcctgtgttctctgtggactatggggagctggatttccagtggcgagagaagaccccggagccccccgtgccctgtgtccctgagcagacggagtatgccaccattgtctttcctagcggaatgggcacctcatcccccgcccgcaggggctcagccgacggccctcggagtgcccagccactgaggcctgaggatggacactgctcttggcccctctgaccggcttccttggccaccagtgttctgcagaccctccaccatgagcccgggtcagcgcatttcctcaggagaagcaggcagggtgcaggccattgcaggccgtccaggggctgagctgcctgggggcgaccggggctccagcctgcacctgcaccaggcacagccccaccacaggactcatgtctcaatgcccacagtgagcccaggcagcaggtgtcaccgtcccctacagggagggccagatgcagtcactgcttcaggtcctgccagcacagagctgcctgcgtccagctccctgaatctctgctgctgctgctgctgctgctgctgctgcctgcggcccggggctgaaggcgccgtggccctgcctgacgccccggagcctcctgcctgaacttgggggctggttggagatggccttggagcagccaaggtgcccctggcagtggcatcccgaaacgccctggacgcagggcccaagactgggcacaggagtgggaggtacatggggctggggactccccaggagttatctgctccctgcaggcctagagaagtttcagggaaggtcagaagagctcctggctgtggtgggcagggcaggaaacccctccacctttacacatgcccaggcagcacctcaggccctttgtggggcagggaagctgaggcagtaagcgggcaggcagagctggaggcctttcaggcccagccagcactctggcctcctgccgccgcattccaccccagcccctcacaccactcgggagagggacatcctacggtcccaaggtcaggagggcagggctggggttgactcaggcccctcccagctgtggccacctgggtgttgggagggcagaagtgcaggcacctagggccccccatgtgcccaccctgggagctctccttggaacccattcctgaaattatttaaaggggttggccgggctcccaccagggcctgggtgggaaggtacaggcgttcccccggggcctagtacccccgccgtggcctatccactcctcacatccacacactgcacccccactcctggggcagggccaccagcatccaggcggccagcaggcacctgagtggctgggacaagggatcccccttccctgtggttctattatattataattataattaaatatgagagcatgctaaggagttctgtcctgtctggtggctgtgggggcagtgggcaggagggagggaggcctccagggagggacaaggcggcagccaggctgaggctgtgtgtggagggtgctggtggctcccctggatcctggcctgagtcaggccttcccctcgctgtcccagaaacacacaggccctcctcgccctgtttgccccactcacatgtagagccctccggtgaaaaattcctccaacatcacggggctggggacaccatcttccccaagcccaggccttttaggggggtcccacggccccctggccccaggcttcctggccaggcatgggtgtccctgagtgactgtgcctgctccatagcccccgtgtccccatgcctaccagtccctccgggcaggggtggtacctggtgccagggcgtccacagcggggtgggagggctgccctgggctatgagggacacagcatctgcgggtccctccccaagtacacagggtgggggcagcgggggaggcggggtcacgtctgctggagccctatcaccctgctgcggtccttggcagctagcagcagggacggtgcagggaaaggagccctgccaggccctcgggcaccgcagccaaacacccactgacaccccggggctcattctctgcttgccatcctg

SEQ ID NO: 2 - DNA, 418 bp, Homo sapiens
ggagagtgaggccaaggcctcccccacggatggtctgaacagggctcggggagagccctggaatctgggcagagacccaggcgggcacaatccccacccaggagggatcctggagacagaagaactgtcctcactcgaacaggtacactttggatataatgagaaaaatatcaccagctcatctaaactttgacgtcgtaaagccaaggttagtcccacatggggctcatcccatccttaggaaaactcgagtgaggaccaaggatgcctgggcaaggcagagccgccacgcagactccccacggccaaggtttggggttctggccagcctgacccgtcattctacagaaacacgcagccccaaggaccggctgagaggggacagaggtcctgcctgcccaggagcaaagaggggact

SEQ ID NO: 3 - DNA, 264 bp, Homo sapiens
gcagggtcaggagggagacagagcccatcccggggctgtggaacaggcctgtgaggtggcggtgggggtgctcccgcagagagaccgcattacaggacattgctttccagaagcgcacagaagaaggctgcctgccccgggcggaggaacctgctggcccagaccagacccggcatctctgaccgtggtcccattagggacaaggaaaccgtcccacgggctgtgctgggatgaggacagcgagcttgtccctagaggacctgg

SEQ ID NO: 4 - DNA, 250 bp, Homo sapiens
ccagaatctccagttctgagtcctgagtgacccacgggccaaccttaagaggtggcgctgaggcaggaaggcacggccctgacaaggatgctgcctcaggtgccggggagcaggccccgggagaggggccgaggtggggaacccccagtcgcctgccacagtgaaggggcaccaggacccccggggcaggagcctcgagggggtgtcagggcggccccaggggtgcccctcatcttgtcctcccagtggt

SEQ ID NO: 5 - DNA, 499 bp, Homo sapiens
cttctggcatcagggccaagagggctcctgggaggcagcctgggacagggtgggctgcagcccttactgggcctaggctggggctgggtggactcggcacagagcaggggaaatgccctgccctctgggtttctgggaatgcagtggggacccaggggccccaccaccgcaggcagcccctcggggtctccatctcccaggccagggctgccatgcagctgtcgggacagacaggcaggtgaggaacagaagtcatcacgggtactgtgagcagggaccctgcatggctaggaagtgctaagggaccccccagctgtagggcgaggtgctggcgacaggacaatggccgctgtgtgtccacaccgcaatgtccctgggaccatctgtgcattgttcttgtaactggaaacttagctgctatttatttgcacacattggtggagggacctgctcctgacttgatctgtgctggcgctgacaggctcaacccttttcctgt

SEQ ID NO: 6 - DNA, 28 bp, Homo sapiens
gtttagattagatttggtatttttgatt

SEQ ID NO: 7 - DNA, 23 bp, Homo sapiens
caaatcctctaaaaacaaactca

SEQ ID NO: 8 - DNA, 27 bp, Homo sapiens
tcccaacacaacccataaaacaatttc

SEQ ID NO: 9 - DNA, 25 bp, Homo sapiens
agattagattcggtatttttgatcg

SEQ ID NO: 10 - DNA, 23 bp, Homo sapiens
caaatcctctaaaaacaaactcg

SEQ ID NO: 11 - DNA, 26 bp, Homo sapiens
cccaacacaacccgtaaaacgatttc

SEQ ID NO: 12 - DNA, 264 bp, Homo sapiens
ttaggttttttagggataagtttgttgtttttattttagtatagtttgtgggatggtttttttgtttttaatgggattatggttagagatgttgggtttggtttgggttagtaggtttttttgtttggggtaggtagtttttttttgtgtgtttttggaaagtaatgttttgtaatgtggtttttttgtgggagtatttttattgttattttataggtttgttttatagttttgggatgggttttgttttttttttgattttgt

SEQ ID NO: 13 - DNA, 264 bp, Homo sapiens
ttaggttttttagggataagttcgttgtttttattttagtatagttcgtgggacggtttttttgtttttaatgggattacggttagagatgtcgggtttggtttgggttagtaggttttttcgttcggggtaggtagtttttttttgtgcgtttttggaaagtaatgttttgtaatgcggtttttttgcgggagtatttttatcgttattttataggtttgttttatagtttcgggatgggttttgttttttttttgattttgt